European Patent Application EP 4 122 954 A1, published January 25, 2023. Title: NOVEL GLP-1 ANALOGUE. Applicant: Sun Pharmaceutical Industries Ltd. The sequence listing filed with the application follows.

SEQUENCE LISTING (14 sequences)

SEQ ID NO: 1 - protein, 31 aa, Homo sapiens
  MISC_FEATURE: Native GLP-1 (7-37)
HAEGTFTSDVSSYLEGQAAKEFIAWLVKGRG

SEQ ID NO: 2 - protein, 31 aa, Artificial Sequence
  Synthetic
  MISC_FEATURE: Liraglutide
  MISC_FEATURE (20)..(20): Lys is substituted
HAEGTFTSDVSSYLEGQAAKEFIAWLVRGRG

SEQ ID NO: 3 - protein, 31 aa, Artificial Sequence
  Synthetic
  MISC_FEATURE: Semaglutide
  MISC_FEATURE (2)..(2): Xaa= Aib
  MISC_FEATURE (20)..(20): Lys is substituted
HXEGTFTSDVSSYLEGQAAKEFIAWLVRGRG

SEQ ID NO: 4 - protein, 34 aa, Artificial Sequence
  Synthetic
  MISC_FEATURE (2)..(2): Xaa=  Ser, Ser(OMe), D-Ser, D-Ser(OMe), Ala or Aib
  MISC_FEATURE (3)..(3): Xaa=  Absent or Gln
  MISC_FEATURE (4)..(4): Xaa=  Glu
  MISC_FEATURE (16)..(16): Xaa=  Glu
  MISC_FEATURE (21)..(21): Lys is substituted
  MISC_FEATURE (24)..(24): Xaa=  Ile
  MISC_FEATURE (33)..(33): Xaa=  Leu, D-Leu, D-Ile or Ile
  MISC_FEATURE (34)..(34): Xaa=  Absent
HXXXGTFTSDVSSYLXGQAAXEFXAWLVRGRGXX

SEQ ID NO: 5 - protein, 32 aa, Artificial Sequence
  Synthetic
  MISC_FEATURE (2)..(2): Xaa = Aib
  MISC_FEATURE (20)..(20): Lys is substituted
HXEGTFTSDVSSYLEGQAAKEFIAWLVRGRGL

SEQ ID NO: 6 - protein, 32 aa, Artificial Sequence; identical to SEQ ID NO: 5
  Synthetic
  MISC_FEATURE (2)..(2): Xaa= Ser(OMe)
  MISC_FEATURE (20)..(20): Lys is substituted

SEQ ID NO: 7 - protein, 33 aa, Artificial Sequence
  Synthetic
  MISC_FEATURE (2)..(2): Xaa = Aib
  MISC_FEATURE (21)..(21): Lys is substituted
HXQEGTFTSDVSSYLEGQAAKEFIAWLVRGRGL

SEQ ID NO: 8 - protein, 32 aa, Artificial Sequence
  Synthetic
  MISC_FEATURE (2)..(2): Xaa = Aib
  MISC_FEATURE (20)..(20): Lys is substituted
  MISC_FEATURE (32)..(32): Xaa= D-Leu
HXEGTFTSDVSSYLEGQAAKEFIAWLVRGRGX

SEQ ID NO: 9 - protein, 32 aa, Artificial Sequence
  Synthetic
  MISC_FEATURE (20)..(20): Lys is substituted
HSEGTFTSDVSSYLEGQAAKEFIAWLVRGRGL

SEQ ID NO: 10 - protein, 32 aa, Artificial Sequence
  Synthetic
  MISC_FEATURE (20)..(20): Lys is substituted
HAEGTFTSDVSSYLEGQAAKEFIAWLVRGRGL

SEQ ID NO: 11 - protein, 32 aa, Artificial Sequence
  Synthetic
  MISC_FEATURE (2)..(2): Xaa = Aib
  MISC_FEATURE (20)..(20): Lys is substituted
HXEGTFTSDVSSYLEGQAAKEFIAWLVRGRGI

SEQ ID NO: 12 - protein, 32 aa, Artificial Sequence; identical to SEQ ID NO: 5
  Synthetic
  MISC_FEATURE (2)..(2): Xaa = D-Ser(OMe)
  MISC_FEATURE (20)..(20): Lys is substituted

SEQ ID NO: 13 - protein, 32 aa, Artificial Sequence; identical to SEQ ID NO: 5
  Synthetic
  MISC_FEATURE (2)..(2): Xaa = D-Ser
  MISC_FEATURE (20)..(20): Lys is substituted

SEQ ID NO: 14 - protein, 33 aa, Artificial Sequence
  Synthetic
  MISC_FEATURE (2)..(2): Xaa = Aib
  MISC_FEATURE (21)..(21): Lys is substituted
  MISC_FEATURE (33)..(33): Xaa = D-Leu
HXQEGTFTSDVSSYLEGQAAKEFIAWLVRGRGX